European Patent Application EP 4 749 655 A2, published May 27, 2026. Title: METHODS AND SYSTEMS FOR DETECTING MICROSATELLITE INSTABILITY OF A CANCER IN A LIQUID BIOPSY ASSAY. Applicant: Tempus AI, Inc. The sequence listing filed with the application follows.

SEQUENCE LISTING (4 sequences)

SEQ ID NO: 1 - DNA, 20 bp, synthetic construct
  misc_feature 1..20: note = Synthetic polynucleotide
  source 1..20: mol_type = other DNA
aaattaaaaaaaaaagaaat

SEQ ID NO: 2 - DNA, 22 bp, synthetic construct
  misc_feature 1..22: note = Synthetic polynucleotide
  source 1..22: mol_type = other DNA
aaattaaaaaaaaaaaagaaat

SEQ ID NO: 3 - DNA, 24 bp, synthetic construct
  misc_feature 1..24: note = Synthetic polynucleotide
  source 1..24: mol_type = other DNA
aaattaaaaaaaaaaaaaagaaat

SEQ ID NO: 4 - DNA, 19 bp, synthetic construct
  misc_feature 1..19: note = Synthetic polynucleotide
  source 1..19: mol_type = other DNA
aaattaaaaaaaaagaaat